European Patent Specification EP 4 313 301 B1, published February 25, 2026. Title: VERWENDUNG VON D-ENANTIOMEREN PEPTIDIDLIGANDEN VON MONOMEREM TAU FÜR DIE THERAPIE VERSCHIEDENER TAUOPATHIEN. Applicant: Forschungszentrum Juelich GmbH. The sequence listing filed with the application follows.

SEQUENCE LISTING (7 sequences)

SEQ ID NO: 1 - protein, 17 aa, Artificial Sequence
  D-Peptide
NEMYLWHWQYPQHLRVG

SEQ ID NO: 2 - protein, 16 aa, Artificial Sequence
  D-Peptide
DGGYQILFKIPGGHIH

SEQ ID NO: 3 - protein, 21 aa, Artificial Sequence
  D-Peptide
NEMYLWHWQYPQHLRVRRRRR

SEQ ID NO: 4 - protein, 21 aa, Artificial Sequence
  D-Peptide
NELYLWHWQYPQHLRVRRRRR

SEQ ID NO: 5 - protein, 21 aa, Artificial Sequence
  D-Peptide
DGGYQILFKIPGGHIHRRRRR

SEQ ID NO: 6 - protein, 21 aa, Artificial Sequence
  D-Peptide
RSSYQILFRIPSSHIHRRRRR

SEQ ID NO: 7 - protein, 18 aa, Artificial Sequence
  D-Peptide
YQILFRIPSSHIHRRRRR